European Patent Application EP 4 803 640 A1, published September 9, 2026. Title: Composition for detecting Staphylococcus epidermidis CICARIA strain and uses thereof. Applicant: 코스맥스 주식회사. The sequence listing filed with the application follows.

SEQUENCE LISTING (3 sequences)

SEQ ID NO: 1 - DNA, 28920 bp, Staphylococcus epidermidis
  source 1..28920: mol_type = genomic DNA
ttcactcaacatttttacacttttcacataatcaaccctttataaatagtttatcaaccctttataaaacattataaggctataagtccccaaatataaagttattcgccataaataaaatacgtcttatcaaagttttatctagggttgatagtttcatcaaaggttcgtaaaaggttgataaacctttgataaccatgcattttctcctttaataaccctatttaaagtgctataatatacttaacatatcaaaagccccccaactactggtaatagtcgggggggctggtaataaaacgttatagcacgtttgtttaatatcaaatttatacttgtattatataatgaataacatcttagtgcaagcgcctaaatctttaaataaatataaagctatataaaaacgttttattacctcttaccaaactaaatttcggaagaggtttttattatgtcaaattttaaaagaattacaatacaagaatttgaacaagaaagattttataaactatataaatttttatttgaagatgattattttagaaagcttagtgactctgcaaaaattgcttactgtatgtttagggatcgattcgaattatctaaaatgaataattggattgatgacaatggtaatgtatatttaatatttactactaaagatttatgtgaacttttaaattgcggaactcaaaaagtaactaaaatcaaaaaagaattagaaaattttaatcttttagaacaagaaagaatgggtttaaacaaaccaaataaaatatatatcctagagcctaaaaaaacttctaaaactgatgatagtaaggaatttcgaaaatcaaaattccagaataatgaaaatcaaaattccagagttttgaaagtcaaaaaacaagaatttcgaaaatcaaaatctaatgatactgaatttaataatactgattatatagagactgattataatgatttgaatgatttgaatgatacaaataataatatttctacaactaataatcattcgaatcattcaaattatcaaaaaaataaatttaataatgatgctttaaaatttcaagtacttgaagaattaccaaatcaaatcaaagattatttaagtaattttgaaatcagagagattcgtattattaagagtgttttacttaaagggaaaaagtcttttaataatacacaagatacatattaccgtttagaagatgttgaatttgagttagtaaatgtcttaaaacgttttaaagcaatgttgctacaaaaaaatgaaacagttgaagccatgcaaggttatttaatgcaatcaattaaagctgaactagaagaaatacatacgttgaatatgcgccgtcaaaatatgccgaaatacaatatatttaatgaataattcaaataatctgataacaacaaagagaattcatcggttaaatcatcaaaaaaatagaagttttgtaatatgttaagtgtgtttatctttggggttttacctatatttgttttgattgctattggtttcttgaactctttttaataaacattcctgcgatatagttatcgattaaaccacaaaatcctataatttctgtgtttttttcgtatacgataatttctgccgttttgaaagattctataacattatcgtaattattaacccaatattcttcgttaataaaattatgggttgctatattagaatttagccagatacttcctaaagtttttaaaatttcttggtcttttttatttaatttacgtatcattttttatcaccttgattttgaaacgagttgaaaacgagtttcttcttgtcttgatgactttagccattgcgaccttcgttgaaggtgcctgatctgtaattatcttttgaggtttaccaaattgtttaatgagacgtttgataaatgcatatcttagatagtagccaacggctacaatgataacatccttgttaaattgtttatatctgaaatagttcatagagaaaactcctttttgttaaatttatactataaattcaactttgtaacagaaccttagtaagcaaacaatttttaataacattaaacgactaaatataaaaacgataaagcaagaaaactcttcatatatcaaagaagatgccgacatagaaaaagttattcaaagagtaaatgcaaataaaaagaaatatggctttgaaagtacaacgagcactgaaaaaagcaatgattcagataatactaattctaaatttgaaaattatattcaattaatagaaacacttaaaaataaaatatctattttaaataataaaattcaaaaacaggaaagttgtcacaaaatgacaatagaattttataggaaagaattacaggaaaggtcgaagctacttaaaaatcagcaaatattgactttagaaagtaataaaaaaattcaaaaattggagtacaaactagaagaagaaaagtaacttaactatacatctaagtttgatactagtaataaacagaccaataatgtacaaaaagctacttttaatgaaaaagatgagaaaataaaaaaacaaatagcaaaagaaaatgaattctttaaggatgataataaatatgaaaaaacaagtaataattctgtgaatagtttagtaaaagaacgtaaaaaagtttttaaaaagtatttttcggtcttttagtgtaatttttcattttggatggatattgaaaaaagcaatgtttaatgataattttaagatgttaatatataagtaagggagaagtgttgaataatacatattaaaaatataggtattataaaagttcaaatgaatggtgaagagatggtgtcaaacgcttctgttgttttttggaaaaaaaaacttctaattattacagcagctcatagtgtttttgattggcattataaaaaattcgcagaatctatatctttttttgactatgaaggaaatgaggttaatatcaacagaattgttctaagtaataattgggttagtgaaggtattttggattttgatactgctatattaattccagataaaacaaatgactgcaattacaataagatatatccaaaattcttttatgataaagaacaaaaaataactgttttatatttgaaggacaaattatttaaaaaaaaattaatgtgtcatgaggctaatactttcgaagactatatatacgaatcgagtatgattggtgtaaatctaaaagctaaagaaggttactctggatctccttggtactataaagatgaaaaaggaacatatcaaataacaaatacaagcctctcttttaaaaaatataaaaaattaacatttgctccatactggggtatgcatatgaaagatatgtttctattttctgaaaatgtaaacaatgttaatgaaaaatatattaatcatatattatattaggaggtgaaataatgaataaaaatagtgtcctaaaattacaaggtatacgcacaaaaaaatctacaaatagccaagcatcaaatgccagtgttatgtgtaaaaaacagagtagtgtaagtgttgttttctgtgtatttccacaaggaaataaataacatttaattaaaagggcctgggacataattcctatcaaaatagccagtaaatgagttttcataaattcatttactggcttctttatttacaatacttcgtattgttggctcgctttcttaggggacagcttcagcctgtagtcttcagcttgtcctgttccctcaagagtctcgccaaaatactttgtattcatatgtaattttacattaaaatactttaaaaaaataaggccctttcgtataatttaataaacatcactaaactaaattaacgaggtgccttatgtataaagattataacatgactcaacttactctaccaatggaaacttcagttcttatccccacaaatgatatttcacgacatgtaaatgatattgtagaaacaattcccgagactgaattcgatgaattcagacatcatcgaggtgcaacatcataccatccaaaaatgatgttaaaagtagttttatatgcctacacccaatctgtgttttcaggacgtaagatagaaaaattactcaatgatagtatccgaatgatgtggctatcacaaaatcaaaagccttcttataaaacgattaatcgatttagagtaaatcccaaagtagatgctttattagaatcattatttattcaatttcatagtcagtgtttgaaacaaaatcttattgatgatcaggccatttttattgatggtacgaaagttgaggcaaatgccaatcgatatacatttgtatggaaaaagagtattcaaaaccatgagtcaagaatgaatgaaaactctaaagcactctatcatgaattggtgataaataaaatcatacctgagattaaaaaagatcatgataatgacttaacaaaagaagaaatagatttgattggtagtcatttagataaagaaatcgaagatttaaaccaacatatcgataatgaaaaatgtactaaaataagaaaacaaatacggctcaaaagaactaaaattaaaaaatacaaaaagcaaattaatgattactctcagcgaaagcataaatacgaagtccaaaaatctattttaaaggatagaaatagttattctaaaacagatcacgatgccacatttatgagaatgaaagaagatcatatgaaaaatggacaacttaaaccggggtataatttacaaatagcgacaaattctcaatttgttttattttatgatgtgtatcaaaatccgactgatacaagaacaatgataccttttttaaatacaatacaagagacctacggtcatttacctgaatatattgtagctgacgcaggttatggtagcgaagccaattatatggcaattatagataattttaatcgaacgccactcataacttatggaatgtttataaaagataaaactaaaaaatataaaagtgacatctttaatactcaaaattgggattatgacgaaattaacgatgaattcatttgtccgaataataaaagactaggatttaaaagatatgcctatcgtcatgataaatatggttttaaacgagactttaaattatatgaatgtgatgattgttcagaatgccctctgaaacaacaatgtatgaacttcaattcaaaaacaaataaaaaaataatgaaaaattataattgggaatattttaaagcccaaattaataaaaagctttcagaaccaaaaacaaaaaccatctacagtcaaagaaaaattgatgtggagcctgtttttggatttatgaaggctattttgggtttcactagaatgtccgttcgagggatagataaagccaaaagagaattaggatttgtgctaatggcacttaatataagaaaagtaacagctcaacgagctgaaaataatcaaaaaaataataaaaaagacaatttctatattatttcaatagaaattgtctttttttacttatcctgggactttatgtcccacactcaatttggagttgttaagtgtggattatagatatgtaaaatatataaataatagtcggtattatacaaaaccttcttatgaaaatgaaggcattataaatttgaaacaagttcctcataattttgaaatagtccaaggagaacattggacaaatgttttcaataatacacaacatctacctaaacaaggatggaaaatacatatatgtacacaactgaaagaggctagaaaaactttagatatagtttctaatcttatgttcaaagaaaatgtatcttttaaatatgtaaaaagtatgcacgaattgatgttaaaagattcaaaatatggagatcggagttcttcggggaagtttattactatttatccatcttcaaatgaacaattcatagatttattaaaaaaattggaacatgagctatctaatcttcctaaagggccgtacattttaaatgataaaagatggtataaaagtaatgtctattttagatatggtggttttatgcctaggacttttagatataatggggagatattagatgctatagaagatccaaatggaaatcttatagaagatcaaagaaagccctattatgtattacctgattttattgaggaacccgaagaaataaaaaaaatgaatttggaagttgatcatgaatataaaagaactcctttagataactacaacataaaagaggctctgcattttagtaatggtggtggggtttatttagcggaacataataaatggggtaatgttgtgttaaaagaaggtcgtccacacacatcgacaggcttcgataatattgatgcttttgaaagagttgaaaacgaagggaaagtattgaagaagcttatgaaagcaaattatccagccaaaatatatgattctttttcagcttgggagcataaatttattgtagaagaatatatcgaaggagattctttgtcgatttggatggttaacaaatatccattttcatcagaatctaataatgaaaattatgtaaaatcttcaattaatatcttaaatcaattaattaaagctataaaagaactccacaatttaaatataggttttggagatcttcaaccagctaatattatagtaagtaaggaagaaaaaataagattaatagattttgaaactgcaggttctattaatgattcattatccagtgtaatgactcctggctttataggtagtcccaaaatgaacaaaggccaaggagactggtttgctgtactaagaattgctaagcaaatgtttattcctataggaagcgtccaagatatttctcataatttggacagtgttcataatagttggattaaatcaacttttggacaagaagctttacatattataaaaaaaatagaaaatatatgcaaatatcaaaattctagaccaatgaaagaatttatcacttctcaaaataaaacagtcagaaattttaatttactatctgttaaagaaaaacttataaattgtataaagaatgatctaagagatgaagaattgcttatgcatggagatataagacagtatgaaatgaattctggtaagtggaatgttttgactggtggatttggtgtgattatggcggttaaaagatctggagaatgggatgaaaaatttgataaatggattaagagtatagattactccaatttggggtatttagaaaatgggttatatactgggaaaataggtatagcaaatgtactaatagaatctggatatataaaagaagcagcaacaataattaaaactattaatattgaagatagcaaccaagatatttcattggcatcaggtttaagcggtttaggtttaggttttttaagtatatattatgagcttaaagaaaatatttatttagatgaaagtaaaaaaataggtgaaatgcttgagaataacttccaagataatacacctgtgtatacttttgattatgatatagttgataaaggattcctaactggttggtcaggtgcttctttatttatgtcatgtttatatagagcaactaataacgaaaaatggttacatctttctcgtaaaatgttgaacaaagagttagaaaagacattatttgatgatactggattatttcaagtagatgacgattttcgtatactgccttatctatctagtggtggcgctggtttagcaatacctatgattgcatatgaaagtatagtaaatgaatcgatatggagaaaagagttagaaggtatatcaaaaatagctaaaagtaaaacatttttcaatggaggattatttcaaggtactaccggtatagtagctataagtaatttattagataactatttaaataaagaagatttgactaagtcttctttatttacattaaatttacatttaattgaaacagaaaattgtatttatttaccaggagattcatgttttagggtttcatctgaccttatgtcaggaactgcaggattgttaacagttgttgacgatattattaataatagttatttttcatggttacctttacttaatatagacaagcttataaatttagataaaattacaaggaggtgaagttggtatatgaaaaatgtattggatttacagcaaatgagaagcaaagctggtaaaaagaagccaacaagaaaacaatctagtactagttggggatgtgctccttctagtaacactagttggtttttctgttaattttgtgtgatattcctgattaaggaggtgagttaactatgaacaaagtattatctttgcaacaagaaacagtttcaaaagaagtacaattaaaagctaaatcttcaaaaagtcaaaactgtaagaatagtagtcattctagctggtttatttgctagaaattaaaagaggcaataagatcgtattaaaaatactatcttattgtctcaatttttatggagttgtttaatttgaacgtatacaatattttaaaaatagctattgataataaaagcaagaaaatttatttggcagttataattatcatttctttaattttcacattagcttctttatatttccctttaataataaaaaatattataacagaacttgaaaaaaataaagtgagtgtttttattatttgctatttaattttgtttttaatattaaggtcagttatggaatctataaatgagtatttaatagctaaacttggaaatatagttataaaagacttacaacaaaatatttatgatcgaatagtaaactatccaatatcatttttcgatgaatataatagtggagacttatcaagtagactagtaaacgatacagaagtaattaaagatttaataacatttcatattcctaaagttattaatggattagttatgattgttggggctgtttgtttaatagtgttattagactggaaattgacagtactaattttacttatatctcctgtaatatttggaattatatttccattaatgaaaaaattagaaaatacaggagagatacaacaaaatgaaatctccaattttatatcaaaaactcaagaaacatttaaaaatattaggatggtaaaagcttctactgcagaacaatctgagagtaaaagcatttctagatacataaataatttatttaaagtaaatttatatgaaagtaaggttatgtctttagtatctcctttagtgaaccttttacttatttttggcttactaattatagctggatatggcgcatatcgaattcaaaatgatactttaactttaagtactcttattgcatttataatttactcattccagttaatgagtcctataagttcaataagtagttttataggagaatatcataaatctaatggagcttttaaaagcttaactgttatccttagtaaggatattgaaaatgctaaaaatacatataaatataattttaagttagaggataaattaatatttgataatgtaagtttagaatttaaagaaaaaaaaatccttgataatatctcttttaaattaaataaaggggagtctcttacaattataggtccttcaggatctggaaaaacaacattattaaatgtaatagaaaaattttattatataaacagtggaagtataactatagatggtatagacattaatgatatcaacactcaaaatttaagatacaatataggattagttagccaagatatacctattataagtggtacaataaaagataatttactatatggattgaataatgtaagtattaccaattttgaaattaaagatattttaaaatctactatgctaaaggatcttgttattaatcaaattgatggtattaatagttatgttggagaaagtggtaatcgtctttcaggcggcgaaaaacaaagaattaatatagggagagtacttttaaaaaatcctaatattattttattagatgaagcaacttcaaatctagataatgaatccaaatctgaaattattaactctatatctgaaataacacaagataaaactgttttaaaaataacacacaatatgcatgagttaaaagaagacgaacaaatattatttatagaaaatgggaaaattatttttaaaggaaaacatggtgagttgctgaaaaacaatgaaagatataaaaaattcattaaaaatgaggcttagtactttacctatagtttaaaataaggtattatactatatacagtagttagtataacttatatgagaggggcattatttaatgaatattcaatttaaaaaaggcgccttggaattattagttttattaattgtaaaacaggaagatcaatatgggtactcattaagtcaaattataactaataggatagctatatctgagggtactatatatcctttgctacgtaagcttgtaagagaagaatatttggaaagttactataccccctctaaagaggggccttcgagaaaatattatagtataactagtaaaggtaatgtacgtttaaatttactactcagagaatggaacaactttactgaagcaataaatatgtttgtgaaagagagtggtcttcatgaataaagaagagtatttaagaataattaaaaaaggaattaagaaagtagatgctaaggaaaaagaagatattttaaatgaatatgaatcgcattttattagtggatataaagataataaggatgatacggaaattattaaagagttaggtaatcctataaaggtagctaaagagataaatgctgtaaattcaatatataaaatagaaaaggaaaaaagtgttaaaagcatattttctgcagcattttctattatgggacttagtatcttcaacttatttttaataataattagtttttttatttttttattactcttaccttttgtactagcttactttattgcagttccaataatgattttttcaccaataatattattagtaatgggttgtataaatggctttgacactattaatacaggagacattttcgaagttattaaaggggtagttttaggaattatattagcctttattggttattttattgctaaatatttcttgaaacttttggttctttatttgaattggaatatagatgtatataaaaaggagaaattaaagtgaaatatatatatatatatttattattgattttttcaattattttagtgagttgctctaattctatagataataataattctaaggaaaatagcgaagataaaatagtagaaaaaccattacctaaaaaaatatttgataagaataaagatggacaatatataacagaaaatgaaattagaaaatcaataaaactgtatttagataaaaatgaagaattatctgaagctagtgaatactatgaagataaaatagattctgaagaatcgctgagtcaaaatgaaattaaaaaacttaagaagttaaataatttaaatcaaaaaaatgatgaaaattttaaaagctatataaaaagcaacaaattacctaaaagttacagaaaagacacagaaagaataagtaaatacatttctcattctaataaatattcccaaaatttggaaaagaaaattgataaaataatagacaaaggtataaatcaaaaaaaagtatcaattaaagatattggaaaaatcgaaaatgatagtacaatagtgaatggaagagagcaatctaaaatagaaaaattcttaaatgaaaaaaatattaaaactaaagcctttaaaaagtaattacttattcatcaactttttatttttacagttagaatcacaataatttaaatcacaaaccacccgtgtgaacgggtggtttgttctacgtttataaacctcttttattggccagcccaaaaggacactgacaggtcagtcaactgcactactttcccatcacaccccctaaaagggtactatttttttcgtctttttttaatttcttctcctgtaaatggacctatgtattcttctattgaaatttgatctgcaacgatattctcttgtaattgattacgaatgtaattttcaattacctttttattgctacctactgtatctacataaaatcttttacaccaaaactatctatttccatatctatattttaaattgacttgtctatcaaaaattattaaaatactttcaccttttaaatatccaacaaataatgatgctcttcatttaggtggaatactcactaacatatgaatatgatttttacatgcttctccttatattatttctatgccttttccttcttctaacatttctgcaactcgataatagataatacgtttttatggatttttagcgttaggagaatacaataaaaggtgccctttatatacacctttttctttcgcaacttgaataccttgtgcttgtctacgtttactttcatttcgttcttgttctgaaaccattgctagtatttgaatgattaggtctttcataaatttatctaataatggattaccgatcacttcattcatcataggtaagctagtaatcatcaattgaacttctttatcttttaaataattaactgtgttaatcacctcatcataattacgacctaaacgatcaatggattctactataaatcgatcccccattctcacaaagttaagtgcttcttgaagtaccggtctattttcaatagatttcccatactgtttttctgtaaatattttttcagcaccaaacgtctttaaattttcaagttgcctttctaaattttgatcgattgatgacactctcgcataaccaataatcattgatttcacctcataattaatatacaccctaatcatacgtttaagttacttgtcactttgcttgatatatgagaattatttaaccttataaatgagaaaaaagcaacgcactttaaataagatacgttgctttttcgattgatgaacacctataattaaactattcatctattatttatgattttttgtatatacaatatttctagtttgttaaagagaattaagaaaataaatctcgaaaataatagagggaaaatcagtttttgatataaaaattatacatgtcaacaataatacaaactataagatgatatcagtatttattatgcatttagaatattaaaattccttcattacactcttggcggtttcacttatcaacttatcatttggcttatcacttttattgtctttattcgtaaaaatgactaaaacaataggttcagattggcccttaggataaacaaaagcaacatcatttctagaagcatatgttattgcttgaccacttttatcagcaaccttatagtcttttggaacaccatctttaattaaagtgtctccgtttttattattaaacattaaatcaagtaagaaatttttattttttttgcttaattttccatttgcgataagtttatttaaagtcttgccgaaagcagcaggcgttgaagtatcttttttgctctttggtgaatagtaatttaattctatctcatatctaactggatttgttacttatctcctagttcttttagatgttgtttaacttttttgattccaccgattcttttataattttattgtttgctgtattatcactatatgtcattgaagcctcaataagttcttttaaagtgatatcttttcctacatatttttctaaaataggagaataagcaactatatcatctttgttaatatgtatttttttatttaacttattataaggtacttgttctaacaaaatagcactatttatcgcttttgaagtcgaagcataggcaaatctcttatctgaattaaattttacttccttaccacttttagtatctaaagcataaacaccaatatgagcattatattttttttctaaatcatttaactcttgggtatgtgaactgtttgaattacatgcaacttaaaactaaagcaattacaattaaaaatattaactttttcaaataaaccctccgatattacagttgtaatttttataaatcaataatattacaattgtaatatcggtgtcaatagtttattataaatatttgaaagaaggtgttgaaatggctaagttattaataatgagcatagtaagcttttgttttatatttctattgttattattttttagtacatattaaaaacgctattttaattatatgttaaattataaagtttggtatctaactcttcttgcaggattaattcctttcattcctattaaattctcttttttaaatttaataatgtgaataatcagcgccacagttgaaagtaagtcacacgacttgaacataacataaataccaccaaacctattcaagagttcacaacagatatccataagtttaattgggattcaattgataatatctgcacagttatttggatagtttttagttatattttaagtttaaatttttgaaagccttattatatcttaaatatttaaagaaacagtcactttatctaaacgaaaatgaaaaaaaataaaatagatacgatacttttcaaccatcaatataaaaaaaatattgtgattcgaaaagcagagactattcaatctccaataactttttggtatgggaaatatattattttgattcctagttcatattttaaaagtgtaattgacaaaagactaaaatatataatattgcatgaatatgctcatgcctaaaaatagagatactttacatttaattatctttaatatcttctctattattatgagttacaatccattagtacatattgtaaaaagaaagataattcatgacaatgaagtagaagccgatagaatttgtccttaataatattaacaaaatgaatttaaaacttatgcggaatctattatggactccgtattaaatgttccattttttaataaaaatatattaagccattcatttaatggtaaagagtcattactcaaaagaagattaattaatataaaagaagccacatctgaaaaaacagtccaaattaattctaatttttatttgtattttttacttttttgctcatggtaattcaaagccagtttttgatggggcaatccataactgattataattataaaaagcccttacacaaacggttaccaaattttagataaaagtaaaatttttggttcaaatagtggatctttcgtcatgtacagcatgaagaaagacaaatactatatttataacgaaaaagaaagtagaaaaaggtattctcctaattcaacttataaaaatttatttagctatgtttggacttgaccgacatatttataaatgatgaaaattcacgtatgtcatgggatcataagcattacccttttgatgcttggaataaggaacaaaatttaaatacagcaatgcaaaattcagttaattggtacttcgaacgtattagcgatcaaataccaaagaactatactgcgactcaactcaagcaattaaattatggtaataaaaatttgggaagttataaaagctattggatggaagatagtttgaaaatatctaatcttgaacaagtaatagtttttaaaaatatgatggaacaaaataaccattttagtaaaaaagcaaagaatcaattatcttcttcattattgattaagaaaaatgaaaagtatgaactgtatgggaaaacaggtacaggtatagtaaacgggaagtataataatgggtggtttgtaggttacgtaattacaaatcatgataagtattatttgctacacatttatcagatggaaagccatctgggaaaaatgctgaattaatcagtgaaaaaatattaaaagaaatgggtgttttaaatggccaataagcaagttgaaatatctatggctgaatgggatgttatgaatataatatggggtaaaaaatcagtatcagctaatgaaattgtagttgaaattcaaaaatataaagaagttagcgataaaacgattagaacattaatcacaagactatataaaaaagagattataaaacgatacaaatcagagaatatttatttttactcatcaaatattaaagaagacgatattaaaatgaaaactgctaaaacttttcttaataaactgtatggggggacatgaaaagtttagtgctgaattttgcgaaaaatgaagaattaaataacaaagaaattgaagaattgcgagacattttaaatgatattagtaaaaagtaattagagatatgtttcaaacataatacatatgtaaactatgcttgactcttattaaattagttttgttaataacatttaaaatatattattaaagatgagagtgtacagaaaataaccattttctgtacactcgttttttatgtctaaataagtatgtattacatagaattatgtgttcaaaaacccaacaaaaaatctatgttcacaaaagaccttgtgattaagttatggtacactgaaggtgtatataggaggtttgtattttgaaaataggttatgcaagagtttcaactggattacaaaatttaaatttacaggaagatcgattaaatacacatggttgtgaaaagatatttaatgaccatatgagtggttcaaaaagtaaaagacctggtttagataaagcaattgaatttgcgaggtcaggagataccattgttgtttggagactagatagactaggacgtaacatggaggatttaatcacattagttaatgaacttaacgaacgaggcgtgagttttcatagtttagaagaaaatataacgatggataaatcaagttctacaggacaattattatttcatttattcgcagcatttgcagaatttgaacgtaatttaattttagaacgttcttcagctggccgaattgcggcacgtgcaagaggaagatatggagggaggcctgaaaaattaaataaacaagatttgaatttacttaagacgctttatgataatggcacacccattaaaacaatagcagaacaatggaaagtttcacgtacaactatttatcgttacctcaataaattggaggacaaggaagatgaaaaacaaggagaagtatctaactaatttttctgaagccaaacgtaaagaagctactcaaaagtacaatataataaaaccttttatcttgggaaatcaatctttatcaagtatttctaaaaataaggacattgcattaagtacactttataggtggaataaattatataaggaagaagggcttactggtctaattcataatacaagagttgataaaggtgatcataaattagaacaaaacataattgacgagattaaacgcctttcactcaagaataaaagaaatagtattgctacaattcataggaaaatcgttaattattgtatagaaaaaaattttgataaaccaagctacaaacaagtttatagtattattaaagcaatgcctaagtctgttattgatttctctcaccaaggtgaaaaatactatcaaaataagtacgatttaatacaaataagagaatcctcaagacccaatgaaatatggcaagccgaccatactttgctagatatttatatattagatcaaacaggtaatattaatagaccctggctaaccattattatggatgactatagtcgcgcaattgcaggatactttataagttttgaagctcctaatgctcaaaatacagcattaacactacaccaagcaatatggaataagaataataccaattggccagtatgtggtatacccgaaaaattctacacagatcacgggagtgactttacctcgcatcacatggaacaagtcgctattgatttgaaaattaacttgatgttttcaaaagttggtgtccctcgtggtcgcggaaaatagaacgtttttttcagacagttaaccaaactttcttagagcaacttcctggatatataaacaataatgatactcctagcgatttaatagattttcaaaatttcgaagaaaaattacgatacttttaattgaagattataatcaaaaagagcatagtgctatccagagcactcctatcaatcggtggaacagtaatcattttttccctaatatgccaagcagtttagaacaacttgatttattattattagaaatacctaaatctagaaaaattcattcagatggcattcattttcaaggctttagatacagtaatacaaacctagctgcttatgtaggtgagtatgtattaattcgttacaatcccaatgatatggctgaaatacgtgttttttatagagatgaatttctttgtacagcaatatctcctgatttagctgattattcaattgatataaaagatatacaacacgcacgtagtcagagagaaaaacacttaaaacaaaatattgctagtccaagcaccactgatttaattaaggaagaaaaaaattatggttattcacctcaagaaacgactaaaaacgtcaaaaaattaaagaggtatcgtaatgactaaacatcagaatttcattgaaacgaaagagtataaacgatttgctgaatttgcgatgcttgtatcaaatatcaatatattgggatctgctatggtcaacctggtgtcggaaaaactttatcttctaggtattacacaaattggaatactattgaaaagcaagttaatcatagagggtgggaagatctagctagtaaaacgactgatgatatattatcggtgaataagatattttatactgcaccggctgaaaaacaaacaagattaagtaatgatctatatagtattagtgcaagtattgatttgggtcaaaaattacacatcgtaaataagtatggtcatgatcatagtaaacattatagtgatatgtttaaatatattgatttaattatagtagatgagattgatcgccttaaagtgcaacatttagagcaattaagagctatttatgatgaacataatttagcaatgatatttattggtatgccaggtatagagaaaaaactatctcgttatcctcaactatattcgcgtataggttttgcacatgaatttgataatctaagtaaagacgagacgcatcatatattagaatataagtggcaagatttaggatttgatctaaaactcgaagattttactgattatgaggcaataacgacgattattaaaattacaaaagggaattttaggctgattcatcgtttatttgcacagatagatagaattatggatataaatggcttagataaaatcagtacagaagttgtagaaacagctagagatagtttagtcataggtattcgttaatagaaaaagcaatgtactttaatataggacattgcttttctcatttaataggtaaaatcattctcatatatcaagtaaagtaacagttactataaattcaataactctctttgtatgattagggtgtacctctattagacatttacgtcgattcttttgtcatgatataattttttgtaagagttaaaaaatatataagatagaaagaggaaatactatgcaatcatttgctaaaataactgcacaaggtacatatgtccctgaaaaagttatggataataatgactttgaaaaaatcgtagagacctctgatgaatggatccaacaaagaacaggtattattgagcgaagaatagctgatgaaaatgaatatactagtgatttaagttataaagctgtattagatttacaagaaaagtatcaagtcgacttaaccgatgtagatatgattattaatacgacgttaactcctgattataaaacacctagtgtagcttcatatgtccaagctcagcttgggttaaaaaatgctggggctattgatattaatgctgcttgcgccggatttacatatggacttaatttagctaatggattgattacatcaggacaaaacaaaaaaattttagtcattggttcagaaacattgtctaaaattacagattataatgatcgaagtacgtgtattttgtttggagacggtgccggtgcatttcttgtagaatatgataaagaagaaatgagttttattgcaagtaatgccggatcagatggcttgaaaggtcataacttatattgcacagaattgtctgaagaaatgttttcagatgatttagaaaatcatggttatatcgttcaaaatggacggggcgtttataaatgggcagtcggtaacgttccaaatataatccatgaagttctaaatcaatcaaattacagtattgaagatttgaattggtttgtaccgcatagtgcgaatgctcgaatgattgaatcgatttgtgaaaaagcaaatattgaaacagataaagcattaaagagtcttaaatactatggtaatacttcatcagcaaccatacctttatcaatcgacctagctataaaagaaggtaaaataaaaaaagatgacttaatcctattagttggatttggtgggggcttggcatatgcatctacacttattagatggactatataattttatgagttctcaattatgcatctttttgcattcctctattaaccagtgttataatatgattaacaagaattctagcgtgaatacaccaatcccctcactacggcaatagtgaggggattttttaggtgtggctatagtcgcctatttatcgttgcgattacgtagccaatgcgtaaataacgcaacaatacaaccactgatgactgtggtcgtgatgtgaacaagaatttctagcatgaataacacctcctctctgcgtctaaatttgacgcctgagagataggcgacctgtatattatatcatctcttaatatacgataatagttaacttccgataagtcattttatgttaaaaactatattaaaataaaactttatattactctctcttttccataaacatttcaataagtacttgatggcgacgtattgcatgatcatactcccctaacaattctcgattcataaattgtataagttcttctacattgccattaacatattgagttataaaatttctatatgcttgttctctaccatttgtacccactttatatgaaatcaataaactgctcagaccataaacgaaatctttattaatttcagaataacgaaatacatttttgacacatttgttttcgatgtcatctaattgttgctttttttgttgataattcaaagtatcatctttcattatctcaggtgtcttatttctaacgcctcgaaattcattctttagtaaagaaatcattctaaaagcttctttctcatttaatttcatctcactgtcacccttctttttgttatgatatttcaacttatttttacctaaccacgttttatataagaatactactagtactgttatttctaatactaatactactggaaatgtagaaagaaatattctaaacggtattaataatttaccaaagtcccatctccataaatcatatagtgcttttaaacatgtaattgcaatatatgtatcagcacctactaatatgataaataatgaccatcttagccacataggaaatactttagtttcttttaatgcatccttattaatactaaaaagtgctacgacatgaggtataaaagtcactcttgactctctttttttaatatcgctaatattctcttcatactctttattttcatcttcatcaacatatataagttttccatcatctttatcttcgactctatcacgaacaatatatttcatctttttattattatgcataagttcaacttcataatatttcttttctttgataaatagggggaataaaaatatagcatataccacattaaacgctgtaaatatgtaaaatgcactccataagtctgattttattgaattaatatttttaacctctgaaaatatttcactaatactcaaaaacatcaatatatctaaaagtataaccaaaccaataaatcttaatatatttttaaatagtctacctaatctttctttattgggattcattatattatttctatcaaccagttttgatataatgattccaaataacggtataacaaatatgcttaaccatctcaatatagtattggcaatttcaaaatattccttgatttccatacctattgacacctcattgttatttatatttaattcattttatgattccaatatagtaaattagaagaacatatgatgtttattcaatggtttctgagtcatatttatcaagttaaatagctaccatttctgttcggataactttatttcaaaaatctatcatctcagtttttcaaactttaatgagtattataccaactaaaaaaatgttttgtcctattccttttgcgctttactacaatatattttcacactactttttcatattaaccgttatcatttaaattaaaacactctcgtctgacatcccatttttaaacttaaaaaatcattttatgctatcaacatgcttccatttttagatccaatttatcgcatctaactttacttttatgatacttttttgagtcacatatcgatgcttgatgatatttttgatattttctttttgaccacaatgatgtctttaacgtcaaactaaaaatccaaaaacgtcatattttttaagtgacttttaaatcaaaaatggtcgtgtttcaatttaaaatatgacacaaatgatgagccgttgagctccttttttgaatcatgatcacttcatttttgaacacataaatcatcaaaaacgcgacgtaaaaatgaataacattgaatgattttaatatcctatttgggttcattcaatgaccttagacattcaaaaaaatggcaataaactatatcaaaaaatagttttttggctcgctcttatcgatcattgattgtcattttttaacttttaaaatcgatcccaaacacacccatacatcgtttcatttgcttcatatatacaaaaaagtatcacacattttttgatttgaatcgcccatttttttatattgaaagtccttttttgacgtcttaacatgtcctcgtttttttctttttcatatgatcactgacgatttcaaccacatctaaaataaaatgccatgatatctcaaacacgccttcaacttttcaaaatagctcgttattcactcctatttttcaaagaaaataagtaatctccaaagcacttttttgtgctccggagctaacttttttatataccgagcaccttttaaaaagttacccggtaaagagcataagggacaacgatgccaccttcggtgtcactcagcatagctgaggtttccttaccgctcgcttcgctcacttgctccaactacgttgagcttagagccccaagggctcagctccaatatctactttcgatattggagctaaaataacccgaaaaagccccggtaacttttttaaccaaaaagtagccaattttaaacaaaattgacaatttccaaattttcaaccgcgccgttatgggctttatgacgtctcggtaactttttaaatcccggtaactttcgttattttaatgcatgtttgttttttgaagatgatgttcgttcaaaaaaattgagacgtttttcaaagttcaaaaccacaggaacgatgaccatcgttctagttgaaacgttgaaattttttcgaatagaggtgaaacaaatggtatatcaacacattaatcagtacttgttcaaacatcaaaaagatcctgtgaaggtcgctatcatatgtcaaaaaatctttgaacatcgtgccacgcaaaatgaaatcacaacgatacaacaactctttcaaaacatctatcgttacctacgtgatgatctcaaattgggtttagagttaaccgttgttgcgctcaatccttatgacttacgtgactattttttaatccaatcgtattactatcatgtcatttaacactgtctcaaaacgacactatttgtcgcgaaacaaatcacaaaaatggtatttaataatcatcttaaacaccataaacatcattcaatttgatacctattttaattttttacagacgacaattcctgtcgtctgttttgcttataataaaaatcataagggggacaatattgtgggaaacaagatccaacgaacattaactatctatactaagttacgtgatcaccgttatgttaatgtgcctttgttggctgaaacatttcacgttcatccacgttcgattcaacgagatttagaagatattcgtgactttttaaacgatcaacatcaacatttattatacgaccatcatacgcaaaattattatatgagtcatcaaaccatgaccgatgatcaagtgacaccgacgagtgtcacatatgaaatgacacatcaactttatcaacaattacaacatcattatcaaacatacgtcctcaaaaatgacgcacacaaaatgcttgtgacattccaaatggccccctcagaagccattcatttttgttttacatatcgtcatgcattacgtttagtgtcacctgacacgctctttgcgcaattcacaaccgaactgattcaactacaaatgatttacatgaaaggagcactttaaggtctatgtttcaatcactcaaacaactcaatcatctccgtttgtatcagaatactcaacaactgaatacttcaagtttcttatattttgttcaatcggtctttcaaatcgtcccacgctggttttggttttatatcatcctcgtatcgattgtttttccatttgagattggcaaagaacctttctttgtcccactctcagcaccacccatcatgacgcaactcgtgcatctatataccttcatcgtcatgatattatccccactcacattaacgtacatccgttttgtgaaatctatcagcttcacacgattttattggggtttagtgaaacatgaagatcgctttactgaacgtcataaccaacggattcgtgaagaaagaggcaaagtctacgccgatgatcgttatgcgtttaactacaatcgtcgcaatggccattggactgcgactaatatagacgctgaaaaacggaatcgtcgtgcagagatgggcaatggtgcttggtttatcgccatggggtacctaggttttcttttattctttgtcggtgcctacatgatcatcatgtattttattatcgtccctgtcgccatcggcgttgtcttacacatgtactacaaatatcaagcgtttcaaaaatagtaaggaggaattagatgtatttaacgctgtctcgattgatggtttatttttgattattaagatcaagtaatcatcaatattattgattcaacaaggagcgattctatgaaaacaaaacaattacttagtacgactgccattgcgggaacacttttattatcgggtttacatgcccctcaggcaaaagctgaaagtaacatcaatggatcaaatgctgttgatattattcaacaagtcgacaaacagcacggcaatcaacctgatttaattcgttatggtcaaccgaaagatcatggtgattattatgaagtgacaaccaataacaaatcaggcgtcggcggtgcaggcatcacacgtctttataaagatggcacagttaaacacagtaccgacagcagtggtcaagattttaaaaccttcggtcattatgaagacacatcatcacacaatcaaaacacaccacaagcagcaacacaacacactgaaacatcacaacatgatacaacagatcaaacattaccagagacaggtcaatctcatactggtataacaacaatggttggcatcgtcgcactgatggcgggtatcggattcatcgctcgccgtacttctcacaaagcttaatacgttgacagagcgatagatcttcatattgaagacctatcgcttctttatatccaaaacacaaaggagttatcacaatgaaaaaatggatctatttactcacatgcatcagcttattattagctggatgtagttttaacaaacatacaaatgaaaaaacgaagcaaccatcagcacaaacgactcagcgtgaccatgatcaaaagcatatgaaccaaacccattttagtgattatattcaaagtaacaaaaatcatattttttacgaacttaataccacacaaatgagttcaacacctttaccaatcaaaggctcaggttcaattaaaaacggtttttctatcaacaataatgacgatcaagaattatttaaagaaatggaattaaaaaatgttattgcgactaaaaatggccagacccgtcactttaatattgatcttcgagaagatgagagttacacatttgacaatttttctaaatacaatgaatcagaggttttaaaaaaggttgagcatatcgaacataatttacttgaagatttaaatactgaaaaaccctctacttacgttgatccaattcaaatattaatgactcaagacaatcaaaataaaggcatcaatatcagttttgatcatcagcatacgctgtcacaaatgaaagaagatcttaaaacagcaccttttaatcatgccatagactataacacgagtattaaacctttcaaatatcatggtaaatattttgcgggcttagctaaaattacttatcacagtacatccgaaggatatattttacaaaaattactcatcactgaggttaaggatgatcatacaatgattacaatagataacgataaagattttgatgatgcgcatacgatgtcttatgaagcaaccgaaaatggtcaagataaaaaagaaaaagaagataaagatatcgatcatttataacagtaataaaaaactaatgacttaggtctcatgacatcaattgtctcaaaagttaaagaattacaatttgatgtatcacaaagactatatattcaaaagcaaacctaatatctttatcttaatcaaaatataaaatccaatgtttcacattctcatcacattaatcaacgtcgtatcacattttggtgatacgacgttgttatatatagggaggtcctttaacatgtatgatcatattcaaacgtatattgaacaaatcagttatgacgtcgttgaggttatcttattgtttgaaaaagtcgaccaaaatcatgccgatatggatgagttaaacacattaaatcggcttgctagagctttttatattgactgtcaaagacacaatctattgacacatactcacccacctacaccattcgaaccttatgagctcatcgaatggtttgtttttcaaagttatgaccgtgaatcacttaggtgccttataggcacctttttatttatcattgttgattatattattgatgggatttattccaattccttgattgtcattgagcctctgaacccttaacaatccccaaaaccatcgaatggtcggtgtcatagctcacgctatgccgacattcgtcgatatagtttagttaagggttcttctcaatgacaatcaattttctcggcataaatggtcactactcaactaaaaagtaaaggaaaaacctttttaaaacaacttcaagttgactgagatgaataacattactttttacaaatagtacataaagatgtataatgaaattaacaaatattaagtacatcaacacaccgaacccccaacctatgtccgtaggttgggggttcttttggtgttggcctgtcgtcttattttttactacgttgctctagccaaaatttaaacaacgtgacaaaacactctactataataggtgctattatcaaaacaaatattaagtacatctctacacctccttctgtcgaaattatcgccagaagttaagacgacttcctaattataacaaaatctctttctactgcacgagtccatataatatataatcaccaagtgtatgcaggcatacaatatacatgcatacataatgcgtgcattatgtatatgcaacatctaaatacgataggtcgtcacaagtaaacaagtttaatagtttacttgtatatttgtttactattaaataagtatacgctatgtgtaacttacataaatatacaaaaccaaaacgtttgaaggctaatgaaaacgtgtcattaagggaatgtataaaagatgaataaacgataattataaggaaaagtcttaaacgttgatttcacagcgtttaagactttattacaagttaacataaaaaggagcgccaagtttacgtacttggcgctcctttttaaatgtaattagtcaccaaacaaacgtctccaaaacccttttttaggtggttgttctactttaacaccatgatcgttctttgtttcttcagatgcattattgtttttaagtaactcatcttcttctaagttgctatcattgctctcttcgggaacctctttatttctatctccaacatcttctgcagtttgattttcgtattgttgattaacatttttaacttcttcagtaaattttgcttcttgcgcattgacattttctctatcattcgtagatggattaaaagaataattaagttgcctttcttcttctaattgattctccaatttttgaatttttttattactttctaaagctaatatttgttgattttcaagtaactttgatctttcctgtaactcttttctatagaattctattgttatttcatgacggctttcttgtttttccatctgactatttaaggtgtcaatttgatttttaagtatttctattatttgagtatcacttttagattcaacattaatattatctgatttattcttttttctatcctctgtattaatttcaaacccatatttctttttattttcattcacccttttaatgattttttctacatcagtatcttctttaatgaatgaggtgttttcctgttttactgtctctatatttagtcgcttaatattattaaaaattgtttgtttactaacctctaattc

SEQ ID NO: 2 - DNA, 23 bp, synthetic construct
  source 1..23: mol_type = other DNA
aatagccaagcatcaaatgccag

SEQ ID NO: 3 - DNA, 22 bp, synthetic construct
  source 1..22: mol_type = other DNA
ggaattatgtcccaggcccttt